European Patent Application EP 4 541 370 A1, published April 23, 2025. Title: 면역활성 부위 융합 단백질을 포함하는 결핵 백신 조성물. Applicant: 주식회사 미코라파. Application KR. The sequence listing filed with the application follows.

SEQUENCE LISTING (112 sequences)

SEQ ID NO: 1 - protein, 647 aa, Mycobacterium tuberculosis
MNAHVEQLEFQAEARQLLDLMVHSVYSNKDAFLRELISNASDALDKLRIEALRNKDLEVDTSDLHIEIDADKAARTLTVRDNGIGMAREEVVDLIGTLAKSGTAELRAQLREAKNAAASEELIGQFGIGFYSSFMVADKVQLLTRKAGESAATRWESSGEGTYTIESVEDAPQGTSVTLHLKPEDAEDDLHDYTSEWKIRNLVKKYSDFIAWPIRMDVERRTPASQEEGGEGGEETVTIETETLNSMKALWARPKEEVSEQEYKEFYKHVAHAWDDPLEIIAMKAEGTFEYQALLFIPSHAPFDLFDRDAHVGIQLYVKRVFIMGDCDQLMPEYLRFVKGVVDAQDMSLNVSREILQQDRQIKAIRRRLTKKVLSTIKDVQSSRPEDYRTFWTQFGRVLKEGLLSDIDNRETLLGISSFVSTYSEEEPTTLAEYVERMKDGQQQIFYATGETRQQLLKSPHLEAFKAKGYEVLLLTDPVDEVWVGMVPEFDGKPLQSVAKGEVDLSSEEDTSEAEREERQKEFADLLTWLQETLSDHVKEVRLSTRLTESPACLITDAFGMTPALARIYRASGQEVPVGKRILELNPSHPLVTGLRQAHQDRADDAEKSLAETAELLYGTALLAEGGALEDPARFAELLAERLARTL

SEQ ID NO: 2 - protein, 245 aa, Mycobacterium tuberculosis
MNAHVEQLEFQAEARQLLDLMVHSVYSNKDAFLRELISNASDALDKLRIEALRNKDLEVDTSDLHIEIDADKAARTLTVRDNGIGMAREEVVDLIGTLAKSGTAELRAQLREAKNAAASEELIGQFGIGFYSSFMVADKVQLLTRKAGESAATRWESSGEGTYTIESVEDAPQGTSVTLHLKPEDAEDDLHDYTSEWKIRNLVKKYSDFIAWPIRMDVERRTPASQEEGGEGGEETVTIETETLN

SEQ ID NO: 3 - protein, 169 aa, Mycobacterium tuberculosis
SMKALWARPKEEVSEQEYKEFYKHVAHAWDDPLEIIAMKAEGTFEYQALLFIPSHAPFDLFDRDAHVGIQLYVKRVFIMGDCDQLMPEYLRFVKGVVDAQDMSLNVSREILQQDRQIKAIRRRLTKKVLSTIKDVQSSRPEDYRTFWTQFGRVLKEGLLSDIDNRETLL

SEQ ID NO: 4 - protein, 234 aa, Mycobacterium tuberculosis
LGISSFVSTYSEEEPTTLAEYVERMKDGQQQIFYATGETRQQLLKSPHLEAFKAKGYEVLLLTDPVDEVWVGMVPEFDGKPLQSVAKGEVDLSSEEDTSEAEREERQKEFADLLTWLQETLSDHVKEVRLSTRLTESPACLITDAFGMTPALARIYRASGQEVPVGKRILELNPSHPLVTGLRQAHQDRADDAEKSLAETAELLYGTALLAEGGALEDPARFAELLAERLARTL

SEQ ID NO: 5 - protein, 402 aa, Mycobacterium tuberculosis
SMKALWARPKEEVSEQEYKEFYKHVAHAWDDPLEIIAMKAEGTFEYQALLFIPSHAPFDLFDRDAHVGIQLYVKRVFIMGDCDQLMPEYLRFVKGVVDAQDMSLNVSREILQQDRQIKAIRRRLTKKVLSTIKDVQSSRPEDYRTFWTQFGRVLKEGLLSDIDNRETLLGISSFVSTYSEEEPTTLAEYVERMKDGQQQIFYATGETRQQLLKSPHLEAFKAKGYEVLLLTDPVDEVWVGMVPEFDGKPLQSVAKGEVDLSSEEDTSEAEREERQKEFADLLTWLQETLSDHVKEVRLSTRLTESPACLITDAFGMTPALARIYRASGQEVPVGKRILELNPSHPLVTGLRQAHQDRADDAEKSLAETAELLYGTALLAEGGALEDPARFAELLAERLARTL

SEQ ID NO: 6 - protein, 95 aa, Mycobacterium tuberculosis
MTEQQWNFAGIEAAASAIQGNVTSIHSLLDEGKQSLTKLAAAWGGSGSEAYQGVQQKWDATATELNNALQNLARTISEAGQAMASTEGNVTGMFA

SEQ ID NO: 7 - protein, 172 aa, Mycobacterium tuberculosis
MKNARTTLIAAAIAGTLVTTSPAGIANADDAGLDPNAAAGPDAVGFDPNLPPAPDAAPVDTPPAPEDAGFDPNLPPPLAPDFLSPPAEEAPPVPVAYSVNWDAIAQCESGGNWSINTGNGYYGGLRFTAGTWRANGGSGSAANASREEQIRVAENVLRSQGIRAWPVCGRRG

SEQ ID NO: 8 - protein, 71 aa, Mycobacterium tuberculosis
ADDAGLDPNAAAGPDAVGFDPNLPPAPDAAPVDTPPAPEDAGFDPNLPPPLAPDFLSPPAEEAPPVPVAYN

SEQ ID NO: 9 - protein, 74 aa, Mycobacterium tuberculosis
VNWDAIAQCESGGNWSINTGNGYYGGLRFTAGTWRANGGSGSAANASREEQIRVAENVLRSQGIRAWPVCGRRG

SEQ ID NO: 10 - protein, 185 aa, Mycobacterium tuberculosis
MIDEALFDAEEKMEKAVAVARDDLSTIRTGRANPGMFSRITIDYYGAATPITQLASINVPEARLVVIKPYEANQLRAIETAIRNSDLGVNPTNDGALIRVAVPQLTEERRRELVKQAKHKGEEAKVSVRNIRRKAMEELHRIRKEGEAGEDEVGRAEKDLDKTTHQYVTQIDELVKHKEGELLEV

SEQ ID NO: 11 - protein, 93 aa, Mycobacterium tuberculosis
MIDEALFDAEEKMEKAVAVARDDLSTIRTGRANPGMFSRITIDYYGAATPITQLASINVPEARLVVIKPYEANQLRAIETAIRNSDLGVNPTN

SEQ ID NO: 12 - protein, 92 aa, Mycobacterium tuberculosis
DGALIRVAVPQLTEERRRELVKQAKHKGEEAKVSVRNIRRKAMEELHRIRKEGEAGEDEVGRAEKDLDKTTHQYVTQIDELVKHKEGELLEV

SEQ ID NO: 13 - protein, 260 aa, Mycobacterium tuberculosis
MPLTPADVHNVAFSKPPIGKRGYNEDEVDAFLDLVENELTRLIEENSDLRQRINELDQELAAGGGAGVTPQATQAIPAYEPEPGKPAPAAVSAGMNEEQALKAARVLSLAQDTADRLTNTAKAESDKMLADARANAEQILGEARHTADATVAEARQRADAMLADAQSRSEAQLRQAQEKADALQADAERKHSEIMGTINQQRAVLEGRLEQLRTFEREYRTRLKTYLESQLEELGQRGSAAPVDSNADAGGFDQFNRGKN

SEQ ID NO: 14 - protein, 90 aa, Mycobacterium tuberculosis
MPLTPADVHNVAFSKPPIGKRGYNEDEVDAFLDLVENELTRLIEENSDLRQRINELDQELAAGGGAGVTPQATQAIPAYEPEPGKPAPAA

SEQ ID NO: 15 - protein, 170 aa, Mycobacterium tuberculosis
VSAGMNEEQALKAARVLSLAQDTADRLTNTAKAESDKMLADARANAEQILGEARHTADATVAEARQRADAMLADAQSRSEAQLRQAQEKADALQADAERKHSEIMGTINQQRAVLEGRLEQLRTFEREYRTRLKTYLESQLEELGQRGSAAPVDSNADAGGFDQFNRGKN

SEQ ID NO: 16 - protein, 295 aa, Mycobacterium tuberculosis
MSKPRKQHGVVVGVDGSLESDAAACWGATDAAMRNIPLTVVHVVNADVATWPPMPYPETWGVWQEDEGRQIVANAVKLAKEAVGADRKLSVKSELVFSTPVPTMVEISNEAEMVVLGSSGRGALARGLLGSVSSSLVRRAGCPVAVIHSDDAVIPDPQHAPVLVGIDGSPVSELATAVAFDEASRRGVELIAVHAWSDVEVVELPGLDFSAVQQEAELSLAERLAGWQERYPDVPVSRVVVCDRPARKLVQKSASAQLVVVGSHGRGGLTGMLLGSVSNAVLHAARVPVIVARQS

SEQ ID NO: 17 - protein, 110 aa, Mycobacterium tuberculosis
MSKPRKQHGVVVGVDGSLESDAAACWGATDAAMRNIPLTVVHVVNADVATWPPMPYPETWGVWQEDEGRQIVANAVKLAKEAVGADRKLSVKSELVFSTPVPTMVEISNE

SEQ ID NO: 18 - protein, 100 aa, Mycobacterium tuberculosis
WSDVEVVELPGLDFSAVQQEAELSLAERLAGWQERYPDVPVSRVVVCDRPARKLVQKSASAQLVVVGSHGRGGLTGMLLGSVSNAVLHAARVPVIVARQS

SEQ ID NO: 19 - protein, 285 aa, Mycobacterium tuberculosis
MTNCAAGKPSSGPNLGRFGSFGRGVTPQQATEIEALGYGAVWVGGSPPAALSWVEPILQATTTLCVATGIVNIWSAPAQRVAESFHRIEAAYPGRFLLGIGVGHAEMISEYRKPYNALVEYLDRLDDYGVPANRRVVAALGPRVLGLSARRSAGAHPYLTTPEHTARARELIGPSAFLAPEHKVVLTTDSARARTVGRQALDMYFNLANYRNNWKRLGFTDDEVSRPGSDRLVDAVVAYGTPDAIAARLNEHLLAGADHVPIQVLTEDDNLVSALTELAKPLRLT

SEQ ID NO: 20 - protein, 138 aa, Mycobacterium tuberculosis
MTNCAAGKPSSGPNLGRFGSFGRGVTPQQATEIEALGYGAVWVGGSPPAALSWVEPILQATTTLCVATGIVNIWSAPAQRVAESFHRIEAAYPGRFLLGIGVGHAEMISEYRKPYNALVEYLDRLDDYGVPANRRVVA

SEQ ID NO: 21 - protein, 147 aa, Mycobacterium tuberculosis
ALGPRVLGLSARRSAGAHPYLTTPEHTARARELIGPSAFLAPEHKVVLTTDSARARTVGRQALDMYFNLANYRNNWKRLGFTDDEVSRPGSDRLVDAVVAYGTPDAIAARLNEHLLAGADHVPIQVLTEDDNLVSALTELAKPLRLT

SEQ ID NO: 22 - protein, 267 aa, Mycobacterium tuberculosis
MYADRDLPGAGGLAVRVIPCLDVDDGRVVKGVNFENLRDAGDPVELAAVYDAEGADELTFLDVTASSSGRATMLEVVRRTAEQVFIPLTVGGGVRTVADVDSLLRAGADKVAVNTAAIACPDLLADMARQFGSQCIVLSVDARTVPVGSAPTPSGWEVTTHGGRRGTGMDAVQWAARGADLGVGEILLNSMDADGTKAGFDLALLRAVRAAVTVPVIASGGAGAVEHFAPAVAAGADAVLAASVFHFRELTIGQVKAALAAEGITVR

SEQ ID NO: 23 - protein, 478 aa, Mycobacterium tuberculosis
MTEKTPDDVFKLAKDEKVEYVDVRFCDLPGIMQHFTIPASAFDKSVFDDGLAFDGSSIRGFQSIHESDMLLLPDPETARIDPFRAAKTLNINFFVHDPFTLEPYSRDPRNIARKAENYLISTGIADTAYFGAEAEFYIFDSVSFDSRANGSFYEVDAISGWWNTGAATEADGSPNRGYKVRHKGGYFPVAPNDQYVDLRDKMLTNLINSGFILEKGHHEVGSGGQAEINYQFNSLLHAADDMQLYKYIIKNTAWQNGKTVTFMPKPLFGDNGSGMHCHQSLWKDGAPLMYDETGYAGLSDTARHYIGGLLHHAPSLLAFTNPTVNSYKRLVPGYEAPINLVYSQRNRSACVRIPITGSNPKAKRLEFRSPDSSGNPYLAFSAMLMAGLDGIKNKIEPQAPVDKDLYELPPEEAASIPQTPTQLSDVIDRLEADHEYLTEGGVFTNDLIETWISFKRENEIEPVNIRPHPYEFALYYDV

SEQ ID NO: 24 - protein, 360 aa, Mycobacterium tuberculosis
MTLTALGMPALRSRTNGIADPRVVPTTGPLVDTFGRVANDLRVSLTDRCNLRCSYCMPERGLRWLPGEQLLRPDELARLIHIAVTRLGVTSVRFTGGEPLLAHHLDEVVAATARLRPRPEISLTTNGVGLARRAGALAEAGLDRVNVSLDSIDRAHFAAITRRDRLAHVLAGLAAAKAAGLTPVKVNAVLDPTTGREDVVDLLRFCLERGYQLRVIEQMPLDAGHSWRRNIALSADDVLAALRPHFRLRPDPAPRGSAPAELWLVDAGPNTPRGRFGVIASVSHAFCSTCDRTRLTADGQIRSCLFSTEETDLRRLLRGGADDDAIEAAWRAAMWSKPAGHGINAPDFIQPDRPMSAIGG

SEQ ID NO: 25 - DNA, 27 bp, synthetic construct
  source 1..27: mol_type = other DNA
catatgaacgcccatgtcgagcagttg

SEQ ID NO: 26 - DNA, 24 bp, synthetic construct
  source 1..24: mol_type = other DNA
aagcttcttcatcgagttgagggt

SEQ ID NO: 27 - DNA, 24 bp, synthetic construct
  source 1..24: mol_type = other DNA
catatgaacctggtcaagaaatac

SEQ ID NO: 28 - DNA, 24 bp, synthetic construct
  source 1..24: mol_type = other DNA
aagcttggcgtagaagatctgttg

SEQ ID NO: 29 - DNA, 24 bp, synthetic construct
  source 1..24: mol_type = other DNA
catatggagggactgctgtcagac

SEQ ID NO: 30 - DNA, 27 bp, synthetic construct
  source 1..27: mol_type = other DNA
aagcttcaaggtacgcgcgagacgttc

SEQ ID NO: 31 - DNA, 27 bp, synthetic construct
  source 1..27: mol_type = other DNA
catatggacgacgcgggcttggaccca

SEQ ID NO: 32 - DNA, 27 bp, synthetic construct
  source 1..27: mol_type = other DNA
aagcttcacgctgtaggccacgggcac

SEQ ID NO: 33 - DNA, 30 bp, synthetic construct
  source 1..30: mol_type = other DNA
catatggtgaactgggacgcgatcgcgcag

SEQ ID NO: 34 - DNA, 27 bp, synthetic construct
  source 1..27: mol_type = other DNA
aagcttgccgcggcggccgcagaccgg

SEQ ID NO: 35 - DNA, 27 bp, synthetic construct
  source 1..27: mol_type = other DNA
catatgattgatgaggctctcttcgac

SEQ ID NO: 36 - DNA, 27 bp, synthetic construct
  source 1..27: mol_type = other DNA
aagcttgttggtgggattcactccaag

SEQ ID NO: 37 - DNA, 27 bp, synthetic construct
  source 1..27: mol_type = other DNA
catatggacggcgcccttattcgcgtg

SEQ ID NO: 38 - DNA, 27 bp, synthetic construct
  source 1..27: mol_type = other DNA
aagcttgacctccagcagctcgccttc

SEQ ID NO: 39 - DNA, 27 bp, synthetic construct
  source 1..27: mol_type = other DNA
catatgtctaaaccccgcaagcagcac

SEQ ID NO: 40 - DNA, 27 bp, synthetic construct
  source 1..27: mol_type = other DNA
aagcttctcgttggagatttcaaccat

SEQ ID NO: 41 - DNA, 27 bp, synthetic construct
  source 1..27: mol_type = other DNA
catatggcagagatggtggtgttgggc

SEQ ID NO: 42 - DNA, 27 bp, synthetic construct
  source 1..27: mol_type = other DNA
aagcttcgcgtgcacggcgatcagttc

SEQ ID NO: 43 - DNA, 27 bp, synthetic construct
  source 1..27: mol_type = other DNA
catatgtggagtgacgtcgaagtggtg

SEQ ID NO: 44 - DNA, 27 bp, synthetic construct
  source 1..27: mol_type = other DNA
aagcttcgactgccgtgccacgatcac

SEQ ID NO: 45 - DNA, 27 bp, synthetic construct
  source 1..27: mol_type = other DNA
catatgaccaattgtgccgccggcaaa

SEQ ID NO: 46 - DNA, 27 bp, synthetic construct
  source 1..27: mol_type = other DNA
aagcttggccaccacccggcggttggc

SEQ ID NO: 47 - DNA, 27 bp, synthetic construct
  source 1..27: mol_type = other DNA
catatggcactgggcccccgggtcctg

SEQ ID NO: 48 - DNA, 27 bp, synthetic construct
  source 1..27: mol_type = other DNA
aagcttagtcagtcggagcggcttcgc

SEQ ID NO: 49 - DNA, 35 bp, synthetic construct
  source 1..35: mol_type = other DNA
aaggagatatacatatgtcgatgaaggcgctgtgg

SEQ ID NO: 50 - DNA, 35 bp, synthetic construct
  source 1..35: mol_type = other DNA
gtgcggccgcaagctttgcgaacatcccagtgacg

SEQ ID NO: 51 - DNA, 18 bp, synthetic construct
  source 1..18: mol_type = other DNA
aagaaggtgctgtccacg

SEQ ID NO: 52 - DNA, 40 bp, synthetic construct
  source 1..40: mol_type = other DNA
aaggagatatacatatgctcggtatttcttcgtttgtctc

SEQ ID NO: 53 - DNA, 34 bp, synthetic construct
  source 1..34: mol_type = other DNA
gtgcggccgcaagctttgcgaacatcccagtgac

SEQ ID NO: 54 - DNA, 31 bp, synthetic construct
  source 1..31: mol_type = other DNA
aaggagatatacatatgtcgatgaaggcgct

SEQ ID NO: 55 - DNA, 18 bp, synthetic construct
  source 1..18: mol_type = other DNA
tgcgaacatcccagtgac

SEQ ID NO: 56 - DNA, 36 bp, synthetic construct
  source 1..36: mol_type = other DNA
gtcactgggatgttcgcagccgacgacgcgggcttg

SEQ ID NO: 57 - DNA, 40 bp, synthetic construct
  source 1..40: mol_type = other DNA
ggtggtggtggtggtgctcgaggttgtaggccacgggcac

SEQ ID NO: 58 - DNA, 27 bp, synthetic construct
  source 1..27: mol_type = other DNA
catatgaacgcccatgtcgagcagttg

SEQ ID NO: 59 - DNA, 29 bp, synthetic construct
  source 1..29: mol_type = other DNA
gaattcggcaaggtacgcgcgagacgttc

SEQ ID NO: 60 - DNA, 25 bp, synthetic construct
  source 1..25: mol_type = other DNA
gaattcgatgaccaattgtgccgcc

SEQ ID NO: 61 - DNA, 24 bp, synthetic construct
  source 1..24: mol_type = other DNA
aagcttagtcagtcggagcggctt

SEQ ID NO: 62 - DNA, 27 bp, synthetic construct
  source 1..27: mol_type = other DNA
aagcttatgacagagcagcagtggaat

SEQ ID NO: 63 - DNA, 27 bp, synthetic construct
  source 1..27: mol_type = other DNA
ctcgagtgcgaacatcccagtgacgtt

SEQ ID NO: 64 - DNA, 27 bp, synthetic construct
  source 1..27: mol_type = other DNA
catatgaacgcccatgtcgagcagttg

SEQ ID NO: 65 - DNA, 29 bp, synthetic construct
  source 1..29: mol_type = other DNA
gaattcggcaaggtacgcgcgagacgttc

SEQ ID NO: 66 - DNA, 28 bp, synthetic construct
  source 1..28: mol_type = other DNA
gaattcgatgacagagcagcagtggaat

SEQ ID NO: 67 - DNA, 27 bp, synthetic construct
  source 1..27: mol_type = other DNA
aagctttgcgaacatcccagtgacgtt

SEQ ID NO: 68 - DNA, 24 bp, synthetic construct
  source 1..24: mol_type = other DNA
aagcttatgaccaattgtgccgcc

SEQ ID NO: 69 - DNA, 26 bp, synthetic construct
  source 1..26: mol_type = other DNA
gcggccgcagtcagtcggagcggctt

SEQ ID NO: 70 - DNA, 32 bp, synthetic construct
  source 1..32: mol_type = other DNA
aaggagatatacatatgtcgatgaaggcgctg

SEQ ID NO: 71 - DNA, 18 bp, synthetic construct
  source 1..18: mol_type = other DNA
caaggtacgcgcgagacg

SEQ ID NO: 72 - DNA, 42 bp, synthetic construct
  source 1..42: mol_type = other DNA
cgtctcgcgcgtaccttggaattcatgacagagcagcagtgg

SEQ ID NO: 73 - DNA, 18 bp, synthetic construct
  source 1..18: mol_type = other DNA
tgcgaacatcccagtgac

SEQ ID NO: 74 - DNA, 42 bp, synthetic construct
  source 1..42: mol_type = other DNA
gtcactgggatgttcgcaaagcttatgaccaattgtgccgcc

SEQ ID NO: 75 - DNA, 35 bp, synthetic construct
  source 1..35: mol_type = other DNA
tgctcgagtgcggccgcagtcagtcggagcggctt

SEQ ID NO: 76 - DNA, 35 bp, synthetic construct
  source 1..35: mol_type = other DNA
gatgttcgcaaagcttatgtggagtgacgtcgaag

SEQ ID NO: 77 - DNA, 18 bp, synthetic construct
  source 1..18: mol_type = other DNA
cgactgccgtgccacgat

SEQ ID NO: 78 - DNA, 36 bp, synthetic construct
  source 1..36: mol_type = other DNA
gcacggcagtcggctagcatgaccaattgtgccgcc

SEQ ID NO: 79 - DNA, 35 bp, synthetic construct; identical to SEQ ID NO: 75
  source 1..35: mol_type = other DNA

SEQ ID NO: 80 - DNA, 35 bp, synthetic construct
  source 1..35: mol_type = other DNA
gatgttcgcaaagcttatggacggcgcccttattc

SEQ ID NO: 81 - DNA, 17 bp, synthetic construct
  source 1..17: mol_type = other DNA
gacctccagcagctcgc

SEQ ID NO: 82 - DNA, 42 bp, synthetic construct
  source 1..42: mol_type = other DNA
gcgagctgctggaggtctctagaatgtggagtgacgtcgaag

SEQ ID NO: 83 - DNA, 24 bp, synthetic construct
  source 1..24: mol_type = other DNA
gctagccgactgccgtgccacgat

SEQ ID NO: 84 - DNA, 35 bp, synthetic construct
  source 1..35: mol_type = other DNA
gcacggcagtcggctagcatggcactgggcccccg

SEQ ID NO: 85 - DNA, 24 bp, synthetic construct
  source 1..24: mol_type = other DNA
tctagacgactgccgtgccacgat

SEQ ID NO: 86 - DNA, 36 bp, synthetic construct
  source 1..36: mol_type = other DNA
gcacggcagtcgtctagaatgtatgccgaccgtgac

SEQ ID NO: 87 - DNA, 24 bp, synthetic construct
  source 1..24: mol_type = other DNA
gctagctcgcacggtgattccttc

SEQ ID NO: 88 - DNA, 35 bp, synthetic construct
  source 1..35: mol_type = other DNA
atcaccgtgcgagctagcatggcactgggcccccg

SEQ ID NO: 89 - DNA, 39 bp, synthetic construct
  source 1..39: mol_type = other DNA
gaaggagatatacatatgaacctggtcaagaaatactcc

SEQ ID NO: 90 - DNA, 39 bp, synthetic construct; identical to SEQ ID NO: 89
  source 1..39: mol_type = other DNA

SEQ ID NO: 91 - DNA, 39 bp, synthetic construct; identical to SEQ ID NO: 89
  source 1..39: mol_type = other DNA

SEQ ID NO: 92 - DNA, 39 bp, synthetic construct; identical to SEQ ID NO: 89
  source 1..39: mol_type = other DNA

SEQ ID NO: 93 - DNA, 39 bp, synthetic construct
  source 1..39: mol_type = other DNA
tggtgctcgagtgcggccgcagtcagtcggagcggcttc

SEQ ID NO: 94 - DNA, 33 bp, synthetic construct
  source 1..33: mol_type = other DNA
gagctgctggaggtcatggtctcggcggggatg

SEQ ID NO: 95 - DNA, 33 bp, synthetic construct; identical to SEQ ID NO: 94
  source 1..33: mol_type = other DNA

SEQ ID NO: 96 - DNA, 36 bp, synthetic construct
  source 1..36: mol_type = other DNA
aaggagatatacatatgattgatgaggctctcttcg

SEQ ID NO: 97 - DNA, 41 bp, synthetic construct
  source 1..41: mol_type = other DNA
gcgagctgctggaggtcgaattcatgtctaaaccccgcaag

SEQ ID NO: 98 - DNA, 24 bp, synthetic construct
  source 1..24: mol_type = other DNA
aagcttcgactgccgtgccacgat

SEQ ID NO: 99 - DNA, 24 bp, synthetic construct
  source 1..24: mol_type = other DNA
aagcttcgactgccgtgccacgat

SEQ ID NO: 100 - DNA, 36 bp, synthetic construct
  source 1..36: mol_type = other DNA
gcacggcagtcgaagcttatgaccaattgtgccgcc

SEQ ID NO: 101 - DNA, 32 bp, synthetic construct
  source 1..32: mol_type = other DNA
aaggagatatacatatgacggaaaagacgccc

SEQ ID NO: 102 - DNA, 18 bp, synthetic construct
  source 1..18: mol_type = other DNA
aacgtcgtagtacagcgc

SEQ ID NO: 103 - DNA, 41 bp, synthetic construct; identical to SEQ ID NO: 97
  source 1..41: mol_type = other DNA

SEQ ID NO: 104 - DNA, 24 bp, synthetic construct
  source 1..24: mol_type = other DNA
aagcttcgactgccgtgccacgat

SEQ ID NO: 105 - DNA, 36 bp, synthetic construct; identical to SEQ ID NO: 100
  source 1..36: mol_type = other DNA

SEQ ID NO: 106 - DNA, 34 bp, synthetic construct
  source 1..34: mol_type = other DNA
aaggagatatacatatgacactgaccgcgctggg

SEQ ID NO: 107 - DNA, 33 bp, synthetic construct
  source 1..33: mol_type = other DNA
cgccgtccatgctagcgccaccgatcgcgctca

SEQ ID NO: 108 - DNA, 36 bp, synthetic construct
  source 1..36: mol_type = other DNA
aaggagatatacatatgtatgccgaccgtgaccttc

SEQ ID NO: 109 - DNA, 34 bp, synthetic construct
  source 1..34: mol_type = other DNA
cgccgtccatgctagctcgcacggtgattccttc

SEQ ID NO: 110 - DNA, 34 bp, synthetic construct
  source 1..34: mol_type = other DNA
gctctgtcatgaattcaacgtcgtagtacagcgc

SEQ ID NO: 111 - DNA, 34 bp, synthetic construct
  source 1..34: mol_type = other DNA
gctctgtcatgaattcgccaccgatcgcgctcat

SEQ ID NO: 112 - DNA, 34 bp, synthetic construct
  source 1..34: mol_type = other DNA
gctctgtcatgaattctcgcacggtgattccttc